European Patent Application EP 4 578 950 A1, published July 2, 2025. Title: ラッカーゼ活性を有するタンパク質. Applicant: 長瀬産業株式会社. The sequence listing filed with the application follows.

SEQUENCE LISTING (25 sequences)

SEQ ID NO: 1 - DNA, 26 bp, synthetic construct
  source 1..26: mol_type = other DNA
tatcgctacgtgactgggtcatggct

SEQ ID NO: 2 - DNA, 36 bp, synthetic construct
  source 1..36: mol_type = other DNA
cgggatcctcgcgctaactcacattaattgcgttgc

SEQ ID NO: 3 - DNA, 1551 bp, Escherichia coli
  source 1..1551: mol_type = genomic DNA
atgcaacgtcgtgatttcttaaaatattccgtcgcgctgggtgtggcttcggctttgccgctgtggagccgcgcagtatttgcggcagaacgcccaacgttaccgatccctgatttgctcacgaccgatgcccgtaatcgcattcagttaactattggcgcaggccagtccacctttggcgggaaaactgcaactacctggggctataacggcaatctgctggggccggcggtgaaattacagcgcggcaaagcggtaacggttgatatctacaaccaactgacggaagagacaacgttgcactggcacgggctggaagtaccgggtgaagtcgacggcggcccgcagggaattattccgccaggtggcaagcgctcggtgacgttgaacgttgatcaacctgccgctacctgctggttccatccgcatcagcacggcaaaaccgggcgacaggtggcgatggggctggctgggctggtggtgattgaagatgacgagatcctgaaattaatgctgccaaaacagtggggtatcgatgatgttccggtgatcgttcaggataagaaatttagcgccgacgggcagattgattatcaactggatgtgatgaccgccgccgtgggctggtttggcgatacgttgctgaccaacggtgcaatctacccgcaacacgctgccccgcgtggttggctgcgcctgcgtttgctcaatggctgtaatgcccgttcgctcaatttcgccaccagcgacaatcgcccgctgtatgtgattgccagcgacggtggtctgctacctgaaccagtgaaggtgagcgaactgccggtgctgatgggcgagcgttttgaagtgctggtggaggttaacgataacaaaccctttgacctggtgacgctgccggtcagccagatggggatggcgattgcgccgtttgataagcctcatccggtaatgcggattcagccgattgctattagtgcctccggtgctttgccagacacattaagtagcctgcctgcgttaccttcgctggaagggctgacggtacgcaagctgcaactctctatggacccgatgctcgatatgatggggatgcagatgctaatggagaaatatggcgatcaggcgatggccgggatggatcacagccagatgatgggccatatggggcacggcaatatgaatcatatgaaccacggcgggaagttcgatttccaccatgccaacaaaatcaacggtcaggcgtttgatatgaacaagccgatgtttgcggcggcgaaagggcaatacgaacgttgggttatctctggcgtgggcgacatgatgctgcatccgttccatatccacggcacgcagttccgtatcttgtcagaaaatggcaaaccgccagcggctcatcgcgcgggctggaaagataccgttaaggtagaaggtaatgtcagcgaagtgctggtgaagtttaatcacgatgcaccgaaagaacatgcttatatggcgcactgccatctgctggagcatgaagatacggggatgatgttagggtttacggtataa

SEQ ID NO: 4 - DNA, 12 bp, synthetic construct
  source 1..12: mol_type = other DNA
aggaggtattat

SEQ ID NO: 5 - DNA, 56 bp, synthetic construct
  source 1..56: mol_type = other DNA
aaaagttgaattcaggaggtattatatgcaacgtcgtgatttcttaaaatattccg

SEQ ID NO: 6 - DNA, 45 bp, synthetic construct
  source 1..45: mol_type = other DNA
cccaagcttttataccgtaaaccctaacatcatccccgtatcttc

SEQ ID NO: 7 - DNA, 28 bp, synthetic construct
  source 1..28: mol_type = other DNA
tggggtatcgatgatgttccggtgatcg

SEQ ID NO: 8 - DNA, 29 bp, synthetic construct
  source 1..29: mol_type = other DNA
gcatccccatcattttgagcatcgggtcc

SEQ ID NO: 9 - DNA, 29 bp, synthetic construct
  source 1..29: mol_type = other DNA
ggacccgatgctcaaaatgatggggatgc

SEQ ID NO: 10 - DNA, 27 bp, synthetic construct
  source 1..27: mol_type = other DNA
gcaatcgccatcttcatctggctgacc

SEQ ID NO: 11 - DNA, 27 bp, synthetic construct
  source 1..27: mol_type = other DNA
ggtcagccagatgaagatggcgattgc

SEQ ID NO: 12 - DNA, 25 bp, synthetic construct
  source 1..25: mol_type = other DNA
ggccatcgccgcagcgccatatttc

SEQ ID NO: 13 - DNA, 25 bp, synthetic construct
  source 1..25: mol_type = other DNA
gaaatatggcgctgcggcgatggcc

SEQ ID NO: 14 - protein, 516 aa, Escherichia coli
  SIGNAL 1..28
MQRRDFLKYSVALGVASALPLWSRAVFAAERPTLPIPDLLTTDARNRIQLTIGAGQSTFGGKTATTWGYNGNLLGPAVKLQRGKAVTVDIYNQLTEETTLHWHGLEVPGEVDGGPQGIIPPGGKRSVTLNVDQPAATCWFHPHQHGKTGRQVAMGLAGLVVIEDDEILKLMLPKQWGIDDVPVIVQDKKFSADGQIDYQLDVMTAAVGWFGDTLLTNGAIYPQHAAPRGWLRLRLLNGCNARSLNFATSDNRPLYVIASDGGLLPEPVKVSELPVLMGERFEVLVEVNDNKPFDLVTLPVSQMGMAIAPFDKPHPVMRIQPIAISASGALPDTLSSLPALPSLEGLTVRKLQLSMDPMLDMMGMQMLMEKYGDQAMAGMDHSQMMGHMGHGNMNHMNHGGKFDFHHANKINGQAFDMNKPMFAAAKGQYERWVISGVGDMMLHPFHIHGTQFRILSENGKPPAAHRAGWKDTVKVEGNVSEVLVKFNHDAPKEHAYMAHCHLLEHEDTGMMLGFTV

SEQ ID NO: 15 - DNA, 27 bp, synthetic construct
  source 1..27: mol_type = other DNA
gcaatcgccatcnncatctggctgacc

SEQ ID NO: 16 - DNA, 27 bp, synthetic construct
  source 1..27: mol_type = other DNA
ggtcagccagatgnngatggcgattgc

SEQ ID NO: 17 - protein, 516 aa, synthetic construct
  VARIANT 360: note = any amino acid other than D
  VARIANT 304: note = any amino acid other than G
  VARIANT 373: note = D may be replaced with any amino acid other than D
  VARIANT 374: note = Q may be replaced with any amino acid other than Q
  SIGNAL 1..28
MQRRDFLKYSVALGVASALPLWSRAVFAAERPTLPIPDLLTTDARNRIQLTIGAGQSTFGGKTATTWGYNGNLLGPAVKLQRGKAVTVDIYNQLTEETTLHWHGLEVPGEVDGGPQGIIPPGGKRSVTLNVDQPAATCWFHPHQHGKTGRQVAMGLAGLVVIEDDEILKLMLPKQWGIDDVPVIVQDKKFSADGQIDYQLDVMTAAVGWFGDTLLTNGAIYPQHAAPRGWLRLRLLNGCNARSLNFATSDNRPLYVIASDGGLLPEPVKVSELPVLMGERFEVLVEVNDNKPFDLVTLPVSQMXMAIAPFDKPHPVMRIQPIAISASGALPDTLSSLPALPSLEGLTVRKLQLSMDPMLXMMGMQMLMEKYGDQAMAGMDHSQMMGHMGHGNMNHMNHGGKFDFHHANKINGQAFDMNKPMFAAAKGQYERWVISGVGDMMLHPFHIHGTQFRILSENGKPPAAHRAGWKDTVKVEGNVSEVLVKFNHDAPKEHAYMAHCHLLEHEDTGMMLGFTV

SEQ ID NO: 18 - protein, 516 aa, synthetic construct
  VARIANT 304: note = G may be replaced with any amino acid other than G
  VARIANT 360: note = any amino acid other than D
  VARIANT 373: note = any amino acid other than D
  VARIANT 374: note = Q may be replaced with any amino acid other than Q
  SIGNAL 1..28
MQRRDFLKYSVALGVASALPLWSRAVFAAERPTLPIPDLLTTDARNRIQLTIGAGQSTFGGKTATTWGYNGNLLGPAVKLQRGKAVTVDIYNQLTEETTLHWHGLEVPGEVDGGPQGIIPPGGKRSVTLNVDQPAATCWFHPHQHGKTGRQVAMGLAGLVVIEDDEILKLMLPKQWGIDDVPVIVQDKKFSADGQIDYQLDVMTAAVGWFGDTLLTNGAIYPQHAAPRGWLRLRLLNGCNARSLNFATSDNRPLYVIASDGGLLPEPVKVSELPVLMGERFEVLVEVNDNKPFDLVTLPVSQMGMAIAPFDKPHPVMRIQPIAISASGALPDTLSSLPALPSLEGLTVRKLQLSMDPMLXMMGMQMLMEKYGXQAMAGMDHSQMMGHMGHGNMNHMNHGGKFDFHHANKINGQAFDMNKPMFAAAKGQYERWVISGVGDMMLHPFHIHGTQFRILSENGKPPAAHRAGWKDTVKVEGNVSEVLVKFNHDAPKEHAYMAHCHLLEHEDTGMMLGFTV

SEQ ID NO: 19 - protein, 516 aa, synthetic construct
  VARIANT 304: note = G may be replaced with any amino acid other than G
  VARIANT 360: note = any amino acid other than D
  VARIANT 373: note = D may be replaced with any amino acid other than D
  VARIANT 374: note = any amino acid other than Q
  SIGNAL 1..28
MQRRDFLKYSVALGVASALPLWSRAVFAAERPTLPIPDLLTTDARNRIQLTIGAGQSTFGGKTATTWGYNGNLLGPAVKLQRGKAVTVDIYNQLTEETTLHWHGLEVPGEVDGGPQGIIPPGGKRSVTLNVDQPAATCWFHPHQHGKTGRQVAMGLAGLVVIEDDEILKLMLPKQWGIDDVPVIVQDKKFSADGQIDYQLDVMTAAVGWFGDTLLTNGAIYPQHAAPRGWLRLRLLNGCNARSLNFATSDNRPLYVIASDGGLLPEPVKVSELPVLMGERFEVLVEVNDNKPFDLVTLPVSQMGMAIAPFDKPHPVMRIQPIAISASGALPDTLSSLPALPSLEGLTVRKLQLSMDPMLXMMGMQMLMEKYGDXAMAGMDHSQMMGHMGHGNMNHMNHGGKFDFHHANKINGQAFDMNKPMFAAAKGQYERWVISGVGDMMLHPFHIHGTQFRILSENGKPPAAHRAGWKDTVKVEGNVSEVLVKFNHDAPKEHAYMAHCHLLEHEDTGMMLGFTV

SEQ ID NO: 20 - protein, 516 aa, synthetic construct; identical to SEQ ID NO: 17
  VARIANT 304: note = K, N, R, V, L, S, Y, C, D, F, P, T, A or H
  VARIANT 373: note = D may be replaced with A.
  VARIANT 374: note = Q may be replaced with A
  VARIANT 360: note = K or S
  SIGNAL 1..28

SEQ ID NO: 21 - protein, 516 aa, synthetic construct
  SIGNAL 1..28
MQRRDFLKYSVALGVASALPLWSRAVFAAERPTLPIPDLLTTDARNRIQLTIGAGQSTFGGKTATTWGYNGNLLGPAVKLQRGKAVTVDIYNQLTEETTLHWHGLEVPGEVDGGPQGIIPPGGKRSVTLNVDQPAATCWFHPHQHGKTGRQVAMGLAGLVVIEDDEILKLMLPKQWGIDDVPVIVQDKKFSADGQIDYQLDVMTAAVGWFGDTLLTNGAIYPQHAAPRGWLRLRLLNGCNARSLNFATSDNRPLYVIASDGGLLPEPVKVSELPVLMGERFEVLVEVNDNKPFDLVTLPVSQMKMAIAPFDKPHPVMRIQPIAISASGALPDTLSSLPALPSLEGLTVRKLQLSMDPMLKMMGMQMLMEKYGAAAMAGMDHSQMMGHMGHGNMNHMNHGGKFDFHHANKINGQAFDMNKPMFAAAKGQYERWVISGVGDMMLHPFHIHGTQFRILSENGKPPAAHRAGWKDTVKVEGNVSEVLVKFNHDAPKEHAYMAHCHLLEHEDTGMMLGFTV

SEQ ID NO: 22 - protein, 516 aa, synthetic construct
  VARIANT 304: note = K, V, L, F, S, N, Y, C, R or D
  SIGNAL 1..28
MQRRDFLKYSVALGVASALPLWSRAVFAAERPTLPIPDLLTTDARNRIQLTIGAGQSTFGGKTATTWGYNGNLLGPAVKLQRGKAVTVDIYNQLTEETTLHWHGLEVPGEVDGGPQGIIPPGGKRSVTLNVDQPAATCWFHPHQHGKTGRQVAMGLAGLVVIEDDEILKLMLPKQWGIDDVPVIVQDKKFSADGQIDYQLDVMTAAVGWFGDTLLTNGAIYPQHAAPRGWLRLRLLNGCNARSLNFATSDNRPLYVIASDGGLLPEPVKVSELPVLMGERFEVLVEVNDNKPFDLVTLPVSQMXMAIAPFDKPHPVMRIQPIAISASGALPDTLSSLPALPSLEGLTVRKLQLSMDPMLKMMGMQMLMEKYGDQAMAGMDHSQMMGHMGHGNMNHMNHGGKFDFHHANKINGQAFDMNKPMFAAAKGQYERWVISGVGDMMLHPFHIHGTQFRILSENGKPPAAHRAGWKDTVKVEGNVSEVLVKFNHDAPKEHAYMAHCHLLEHEDTGMMLGFTV

SEQ ID NO: 23 - protein, 516 aa, synthetic construct
  VARIANT 304: note = V, P, T, N, R, H, A, L, F, C or D
  SIGNAL 1..28
MQRRDFLKYSVALGVASALPLWSRAVFAAERPTLPIPDLLTTDARNRIQLTIGAGQSTFGGKTATTWGYNGNLLGPAVKLQRGKAVTVDIYNQLTEETTLHWHGLEVPGEVDGGPQGIIPPGGKRSVTLNVDQPAATCWFHPHQHGKTGRQVAMGLAGLVVIEDDEILKLMLPKQWGIDDVPVIVQDKKFSADGQIDYQLDVMTAAVGWFGDTLLTNGAIYPQHAAPRGWLRLRLLNGCNARSLNFATSDNRPLYVIASDGGLLPEPVKVSELPVLMGERFEVLVEVNDNKPFDLVTLPVSQMXMAIAPFDKPHPVMRIQPIAISASGALPDTLSSLPALPSLEGLTVRKLQLSMDPMLSMMGMQMLMEKYGDQAMAGMDHSQMMGHMGHGNMNHMNHGGKFDFHHANKINGQAFDMNKPMFAAAKGQYERWVISGVGDMMLHPFHIHGTQFRILSENGKPPAAHRAGWKDTVKVEGNVSEVLVKFNHDAPKEHAYMAHCHLLEHEDTGMMLGFTV

SEQ ID NO: 24 - DNA, 29 bp, synthetic construct
  source 1..29: mol_type = other DNA
gcatccccatcatcgagagcatcgggtcc

SEQ ID NO: 25 - DNA, 29 bp, synthetic construct
  source 1..29: mol_type = other DNA
ggacccgatgctctcgatgatggggatgc